European Patent Application EP 4 487 867 A1, published January 8, 2025. Title: IL2突变体-抗体Fc嵌段融合蛋白的药物组合物及其应用. Applicant: 海南先声药业有限公司. The sequence listing filed with the application follows.

SEQUENCE LISTING (20 sequences)

SEQ ID NO: 1 - protein, 133 aa, synthetic construct
APTSSSTKKTQLQLEHLLLDLQMILNGINNYKNPKLTRMLTFKFYMPKKATELKHLQCLEEELKPLEEVLNLAQSKNFHLRPRDLISNINVIVLELKGSETTFMCEYADETATIVEFLNRWITFXQSIISTLT

SEQ ID NO: 2 - protein, 133 aa, synthetic construct
APTSSSTKKTQLQLEHLLLDLQMILNGINNYKNPKLTRMLTFKFYMPKKATELKHLQCLEEELKPLEEVLNLAQSKNFHLRPRDLISNINVIVLELKGSETTFMCEYADETATIVEFLNRWITFAQSIISTLT

SEQ ID NO: 3 - protein, 133 aa, synthetic construct
APTSSSTKKTQLQLEHLLLDLQMILNGINNVKNPKLTRMLTFKFYMPKKATELKHLQCLEEELKPLEEVLNLLQSKNFQLRPRDLISNINVIVLELKGSETTFMCEYADETATIVEFLNRWITFAQSIISTLT

SEQ ID NO: 4 - protein, 133 aa, synthetic construct
APTSSSTKKTQLQLEHLLLDLQMILNGINNYKNPKLTRMLTFKFYMPKKATELKHLQCLEEELKPLEEVLNLAQSKNFHLRPRDLISNINRIVLELKGSETTFMCEYADETATIVEFLNRWITFAQSIISTLT

SEQ ID NO: 5 - protein, 133 aa, synthetic construct
APTSSSTKKTQLQLEELLLDLQMILNGINNYKNPKLTRMLTFKFYMPKKATELKHLQCLEEELKPLEEVLNLAQSKNFHLRPRDLISNINVIVLELKGSETTFMCEYADETATIVEFLNRWITFAQSIISTLT

SEQ ID NO: 6 - protein, 133 aa, synthetic construct
APTSSSTKKTQLQLEHLLLALQMILNGINNYKNPKLTRMLTFKFYMPKKATELKHLQCLEEELKPLEEVLNLAQSKNFHLRPRDLISNINVIVLELKGSETTFMCEYADETATIVEFLNRWITFAQSIISTLT

SEQ ID NO: 7 - protein, 133 aa, synthetic construct
APTSSSTKKTQLQLEELLLDLQMILNGINNYKNPKLTRMLTFKFYMPKKATELKHLQCLEEELKPLEEVLNLAQSKNFHLRPRDLISNINRIVLELKGSETTFMCEYADETATIVEFLNRWITFAQSIISTLT

SEQ ID NO: 8 - protein, 133 aa, synthetic construct
APTSSSTKKTQLQLEHLLLDLQMILNGINNVKNPKLTRMLTFKFYMPKKATELKHLQCLEEELKPLEEVLNLLQSKNFQLRPRDLISNINRIVLELKGSETTFMCEYADETATIVEFLNRWITFAQSIISTLT

SEQ ID NO: 9 - protein, 133 aa, synthetic construct
APTSSSTKKTQLQLEELLLDLQMILNGINNVKNPKLTRMLTFKFYMPKKATELKHLQCLEEELKPLEEVLNLLQSKNFQLRPRDLISNINVIVLELKGSETTFMCEYADETATIVEFLNRWITFAQSIISTLT

SEQ ID NO: 10 - protein, 133 aa, synthetic construct
APTSSSTKKTQLQLEHLLLALQMILNGINNVKNPKLTRMLTFKFYMPKKATELKHLQCLEEELKPLEEVLNLLQSKNFQLRPRDLISNINVIVLELKGSETTFMCEYADETATIVEFLNRWITFAQSIISTLT

SEQ ID NO: 11 - protein, 133 aa, synthetic construct
APTSSSTKKTQLQLEELLLDLQMILNGINNVKNPKLTRMLTFKFYMPKKATELKHLQCLEEELKPLEEVLNLLQSKNFQLRPRDLISNINRIVLELKGSETTFMCEYADETATIVEFLNRWITFAQSIISTLT

SEQ ID NO: 12 - protein, 15 aa, synthetic construct
GGGGSGGGGSGGGGS

SEQ ID NO: 13 - protein, 232 aa, synthetic construct
EPKSSDKTHTCPPCPAPELLGGPSVFLFPPKPKDTLMISRTPEVTCVVVDVSHEDPEVKFNWYVDGVEVHNAKTKPREEQYGSTYRVVSVLTVLHQDWLNGKEYKCKVSNKALPAPIEKTISKAKGQPREPQVYTLPPSRDELTKNQVSLTCLVKGFYPSDIAVEWESNGQPENNYKTTPPVLDSDGSFFLYSKLTVDKSRWQQGNVFSCSVMHEALHNHYTQKSLSLSPGK

SEQ ID NO: 14 - protein, 380 aa, synthetic construct
APTSSSTKKTQLQLEHLLLDLQMILNGINNVKNPKLTRMLTFKFYMPKKATELKHLQCLEEELKPLEEVLNLLQSKNFQLRPRDLISNINVIVLELKGSETTFMCEYADETATIVEFLNRWITFAQSIISTLTGGGGSGGGGSGGGGSEPKSSDKTHTCPPCPAPELLGGPSVFLFPPKPKDTLMISRTPEVTCVVVDVSHEDPEVKFNWYVDGVEVHNAKTKPREEQYGSTYRVVSVLTVLHQDWLNGKEYKCKVSNKALPAPIEKTISKAKGQPREPQVYTLPPSRDELTKNQVSLTCLVKGFYPSDIAVEWESNGQPENNYKTTPPVLDSDGSFFLYSKLTVDKSRWQQGNVFSCSVMHEALHNHYTQKSLSLSPGK

SEQ ID NO: 15 - protein, 380 aa, synthetic construct
APTSSSTKKTQLQLEHLLLDLQMILNGINNVKNPKLTRMLTFKFYMPKKATELKHLQCLEEELKPLEEVLNLLQSKNFQLRPRDLISNINRIVLELKGSETTFMCEYADETATIVEFLNRWITFAQSIISTLTGGGGSGGGGSGGGGSEPKSSDKTHTCPPCPAPELLGGPSVFLFPPKPKDTLMISRTPEVTCVVVDVSHEDPEVKFNWYVDGVEVHNAKTKPREEQYGSTYRVVSVLTVLHQDWLNGKEYKCKVSNKALPAPIEKTISKAKGQPREPQVYTLPPSRDELTKNQVSLTCLVKGFYPSDIAVEWESNGQPENNYKTTPPVLDSDGSFFLYSKLTVDKSRWQQGNVFSCSVMHEALHNHYTQKSLSLSPGK

SEQ ID NO: 16 - protein, 380 aa, synthetic construct
APTSSSTKKTQLQLEELLLDLQMILNGINNVKNPKLTRMLTFKFYMPKKATELKHLQCLEEELKPLEEVLNLLQSKNFQLRPRDLISNINVIVLELKGSETTFMCEYADETATIVEFLNRWITFAQSIISTLTGGGGSGGGGSGGGGSEPKSSDKTHTCPPCPAPELLGGPSVFLFPPKPKDTLMISRTPEVTCVVVDVSHEDPEVKFNWYVDGVEVHNAKTKPREEQYGSTYRVVSVLTVLHQDWLNGKEYKCKVSNKALPAPIEKTISKAKGQPREPQVYTLPPSRDELTKNQVSLTCLVKGFYPSDIAVEWESNGQPENNYKTTPPVLDSDGSFFLYSKLTVDKSRWQQGNVFSCSVMHEALHNHYTQKSLSLSPGK

SEQ ID NO: 17 - protein, 380 aa, synthetic construct
APTSSSTKKTQLQLEHLLLALQMILNGINNVKNPKLTRMLTFKFYMPKKATELKHLQCLEEELKPLEEVLNLLQSKNFQLRPRDLISNINVIVLELKGSETTFMCEYADETATIVEFLNRWITFAQSIISTLTGGGGSGGGGSGGGGSEPKSSDKTHTCPPCPAPELLGGPSVFLFPPKPKDTLMISRTPEVTCVVVDVSHEDPEVKFNWYVDGVEVHNAKTKPREEQYGSTYRVVSVLTVLHQDWLNGKEYKCKVSNKALPAPIEKTISKAKGQPREPQVYTLPPSRDELTKNQVSLTCLVKGFYPSDIAVEWESNGQPENNYKTTPPVLDSDGSFFLYSKLTVDKSRWQQGNVFSCSVMHEALHNHYTQKSLSLSPGK

SEQ ID NO: 18 - protein, 380 aa, synthetic construct
APTSSSTKKTQLQLEELLLDLQMILNGINNVKNPKLTRMLTFKFYMPKKATELKHLQCLEEELKPLEEVLNLLQSKNFQLRPRDLISNINRIVLELKGSETTFMCEYADETATIVEFLNRWITFAQSIISTLTGGGGSGGGGSGGGGSEPKSSDKTHTCPPCPAPELLGGPSVFLFPPKPKDTLMISRTPEVTCVVVDVSHEDPEVKFNWYVDGVEVHNAKTKPREEQYGSTYRVVSVLTVLHQDWLNGKEYKCKVSNKALPAPIEKTISKAKGQPREPQVYTLPPSRDELTKNQVSLTCLVKGFYPSDIAVEWESNGQPENNYKTTPPVLDSDGSFFLYSKLTVDKSRWQQGNVFSCSVMHEALHNHYTQKSLSLSPGK

SEQ ID NO: 19 - protein, 380 aa, synthetic construct
APTSSSTKKTQLQLEHLLLDLQMILNGINNYKNPKLTRMLTFKFYMPKKATELKHLQCLEEELKPLEEVLNLAQSKNFHLRPRDLISNINVIVLELKGSETTFMCEYADETATIVEFLNRWITFAQSIISTLTGGGGSGGGGSGGGGSEPKSSDKTHTCPPCPAPELLGGPSVFLFPPKPKDTLMISRTPEVTCVVVDVSHEDPEVKFNWYVDGVEVHNAKTKPREEQYGSTYRVVSVLTVLHQDWLNGKEYKCKVSNKALPAPIEKTISKAKGQPREPQVYTLPPSRDELTKNQVSLTCLVKGFYPSDIAVEWESNGQPENNYKTTPPVLDSDGSFFLYSKLTVDKSRWQQGNVFSCSVMHEALHNHYTQKSLSLSPGK

SEQ ID NO: 20 - protein, 368 aa, synthetic construct
PKSSDKTHTCPPCPAPELLGGPSVFLFPPKPKDTLMISRTPEVTCVVVDVSHEDPEVKFNWYVDGVEVHNAKTKPCEEQYGSTYRCVSVLTVLHQDWLNGKEYKCKVSNKALPAPIEKTISKAKGQPREPQVYTLPPSRDELTKNQVSLTCLVKGFYPSDIAVEWESNGQPENNYKTTPPVLDSDGSFFLYSKLTVDKSRWQQGNVFSCSVMHEALHNHYTQKSLSLSPGGGGGSAPTSSSTKKTQLQLEHLLLDLQMILNGINNYKNPKLTRMLTFKFYMPKKATELKHLQCLEEELKPLEEVLNLAQSKNFHLRPRDLISNINKIVLELKGSETTFMCEYADETATIVEFLNRWITFAQSIISTLT